European Patent Application EP 4 119 152 A1, published January 18, 2023. Title: IFN-γ在制备抗肿瘤辅助药物中的应用. Applicant: 四川大学华西医院. The sequence listing filed with the application follows.

SEQUENCE LISTING (3 sequences)

SEQ ID NO: 1 - DNA, 1425 bp, Artificial sequence
atggccttaccagtgaccgccttgctcctgccgctggccttgctgctccacgccgccaggccgatgcaggtacaactgcagcagtcaggacctgaactgaagaagcctggagagacagtcaagatctcctgcaaggcctctgggtatcctttcacaaactatggaatgaactgggtgaagcaggctccaggacagggtttaaagtggatgggctggattaacacctccactggagagtcaacatttgctgatgacttcaagggacggtttgacttctctttggaaacctctgccaacactgcctatttgcagatcaacaacctcaaaagtgaagactcggctacatatttctgtgcaagatgggaggtttaccacggctacgttccttactggggccaagggaccacggtcaccgtttcctctggcggtggcggttctggtggcggtggctccggcggtggcggttctgacatccagctgacccagtctcacaaattcctgtccacttcagtaggagacagggtcagcatcacctgcaaggccagtcaggatgtgtataatgctgttgcctggtatcaacagaaaccaggacaatctcctaaacttctgatttactcggcatcctcccggtacactggagtcccttctcgcttcactggcagtggctctgggccggatttcactttcaccatcagcagtgtgcaggctgaagacctggcagtttatttctgtcagcaacattttcgtactccattcacgttcggctcggggacaaaattggagatcaaaaccacgacgccagcgccgcgaccaccaacaccggcgcccaccatcgcgtcgcagcccctgtccctgcgcccagaggcgtgccggccagcggcggggggcgcagtgcacacgagggggctggacttcgcctgtgatatctacatctgggcgcccctggccgggacttgtggggtccttctcctgtcactggttatcaccaaacggggcagaaagaaactcctgtatatattcaaacaaccatttatgagaccagtacaaactactcaagaggaagatggctgtagctgccgatttccagaagaagaagaaggaggatgtgaactggcccccgcgtaccagcagggccagaaccagctctataacgagctcaatctaggacgaagagaggagtacgatgttttggacaagagacgtggccgggaccctgagatggggggaaagccgcagagaaggaagaaccctcaggaaggcctgtacaatgaactgcagaaagataagatggcggaggcctacagtgagattgggatgaaaggcgagcgccggaggggcaaggggcacgatggcctttaccagggtctcagtacagccaccaaggacacctacgacgcccttcacatgcaggccctgccccctcgc

SEQ ID NO: 2 - DNA, 501 bp, Artificial sequence
atgaaatatacaagttatatcttggcttttcagctctgcatcgttttgggttctcttggctgttactgccaggacccatatgtaaaagaagcagaaaaccttaagaaatattttaatgcaggtcattcagatgtagcggataatggaactcttttcttaggcattttgaagaattggaaagaggagagtgacagaaaaataatgcagagccaaattgtctccttttacttcaaactttttaaaaactttaaagatgaccagagcatccaaaagagtgtggagaccatcaaggaagacatgaatgtcaagtttttcaatagcaacaaaaagaaacgagatgacttcgaaaagctgactaattattcggtaactgacttgaatgtccaacgcaaagcaatacatgaactcatccaagtgatggctgaactgtcgccagcagctaaaacagggaagcgaaaaaggagtcagatgctgtttcgaggtcgaagagcatcccagtaa

SEQ ID NO: 3 - DNA, 66 bp, Artificial sequence
ggaagcggagctactaacttcagcctgctgaagcaggctggagacgtggaggagaaccctggacct